European Patent Specification EP 3 639 832 B1, published April 3, 2024. Title: A composition comprising an exosome derived from adipose-derived stem cell as an active ingredient and its application for improving dermatitis. Applicant: ExoCoBio Inc. The sequence listing filed with the application follows.

SEQUENCE LISTING (28 sequences)

SEQ ID NO: 1 - DNA, 24 bp, Artificial Sequence
  TNF-alpha forward primer
tctcatcagttctatggcccagac

SEQ ID NO: 2 - DNA, 24 bp, Artificial Sequence
  TNF-alpha reverse primer
ggcaccactagttggttgtctttg

SEQ ID NO: 3 - DNA, 24 bp, Artificial Sequence
  iNOS forward primer
gctaccacattgaagaagctggtg

SEQ ID NO: 4 - DNA, 24 bp, Artificial Sequence
  iNOS reverse primer
ccataggaaaagactgcaccgaag

SEQ ID NO: 5 - DNA, 24 bp, Artificial Sequence
  GAPDH forward primer
gacatcaagaaggtggtgaagcag

SEQ ID NO: 6 - DNA, 24 bp, Artificial Sequence
  GAPDH reverse primer
ccctgttgctgtagccgtattcat

SEQ ID NO: 7 - DNA, 24 bp, Artificial Sequence
  IL-6 forward primer
gccagagtccttcagagagataca

SEQ ID NO: 8 - DNA, 24 bp, Artificial Sequence
  IL-6 reverse primer
attggatggtcttggtccttagcc

SEQ ID NO: 9 - DNA, 24 bp, Artificial Sequence
  IL-1beta forward primer
gcaacgacaaaatacctgtggcct

SEQ ID NO: 10 - DNA, 24 bp, Artificial Sequence
  IL-1beta reverse primer
agttggggaactctgcagactcaa

SEQ ID NO: 11 - DNA, 19 bp, Artificial Sequence
  IL-4 forward primer
acaggagaagggacgccat

SEQ ID NO: 12 - DNA, 21 bp, Artificial Sequence
  IL-4 reverse primer
gaagccctacagacgagctca

SEQ ID NO: 13 - DNA, 20 bp, Artificial Sequence
  IL-31 forward primer
cacacaggaacaacgaagcc

SEQ ID NO: 14 - DNA, 19 bp, Artificial Sequence
  IL-31 reverse primer
cgatattggggcaccgaag

SEQ ID NO: 15 - DNA, 20 bp, Artificial Sequence
  IL-23 forward primer
cacatgcaccagcgggacat

SEQ ID NO: 16 - DNA, 24 bp, Artificial Sequence
  IL-23 reverse primer
ctttgcaagcagaactggctgttg

SEQ ID NO: 17 - DNA, 20 bp, Artificial Sequence
  TNF-alpha forward primer
cgtcgtagcaaaccaccaag

SEQ ID NO: 18 - DNA, 24 bp, Artificial Sequence
  TNF-alpha reverse primer
ttgaagagaacctgggagtagaca

SEQ ID NO: 19 - DNA, 20 bp, Artificial Sequence
  GAPDH forward primer
catggccttccgtgttccta

SEQ ID NO: 20 - DNA, 22 bp, Artificial Sequence
  GAPDH reverse primer
cctgcttcaccaccttcttgat

SEQ ID NO: 21 - DNA, 24 bp, Artificial Sequence
  IL-6 (THP-1) forward primer
aagccagagctgtgcagatgagta

SEQ ID NO: 22 - DNA, 20 bp, Artificial Sequence
  IL-6 (THP-1) reverse primer
tgtcctgcagccactggttc

SEQ ID NO: 23 - DNA, 24 bp, Artificial Sequence
  IL-1beta (THP-1) forward primer
acctgtcctgcgtgttgaaagatg

SEQ ID NO: 24 - DNA, 24 bp, Artificial Sequence
  IL-1beta (THP-1) reverse primer
tgggcagactcaaattccagcttg

SEQ ID NO: 25 - DNA, 20 bp, Artificial Sequence
  TNF-alpha (THP-1) forward primer
ctgcctgctgcactttggag

SEQ ID NO: 26 - DNA, 23 bp, Artificial Sequence
  TNF-alpha (THP-1) reverse primer
acatgggctacaggcttgtcact

SEQ ID NO: 27 - DNA, 22 bp, Artificial Sequence
  GAPDH (THP-1) forward primer
ctttggtatcgtggaaggactc

SEQ ID NO: 28 - DNA, 22 bp, Artificial Sequence
  GAPDH (THP-1) reverse primer
gtagaggcagggatgatgttct